European Patent Application EP 4 151 724 A1, published March 22, 2023. Title: METHOD FOR INDUCING GLIAL CELLS TRANSDIFFERENTIATION INTO FUNCTIONAL NEURONS, AND APPLICATION THEREOF. Applicant: NEURAGEN BIOTHERAPEUTICS (SUZHOU) CO., LTD. Application EP21805293.4. The sequence listing filed with the application follows.

SEQUENCE LISTING (6 sequences)

SEQ ID NO: 1 - protein, 263 aa, Mus musculus
MFVKSETLELKEEEEVLMLLGSASPASATLTPMSSSADEEEDEELRRPGSARGQRGAEAEQGVQGSPASGAGGCRPGRLLGLMHECKRRPSRSRAVSRGAKTAETVQRIKKTRRLKANNRERNRMHNLNAALDALREVLPTFPEDAKLTKIETLRFAHNYIWALTETLRLADHCAGAGGLQGALFTEAVLLSPGAALGASGDSPSPPSSWSCTNSPASSSNSTSPYSCTLSPASPGSDVDYWQPPPPEKHRYAPHLPLARDCI

SEQ ID NO: 2 - DNA, 792 bp, Mus musculus
atgttcgtcaaatctgagactctggagttgaaggaggaagaggaggtactgatgctgctgggctcggcttccccggcctcggcgaccctgaccccgatgtcctccagcgcggacgaggaggaggacgaggagctgcgccggccgggctccgcgcgtgggcagcgtggagcggaagccgagcagggggtgcagggcagtccggcgtcgggtgccgggggttgccggccagggcggctgctgggcctgatgcacgagtgcaagcgtcgcccgtcgcgctcacgggccgtctcccgaggtgccaagacggcggagacggtgcagcgcatcaagaagacccgcaggctcaaggccaacaaccgcgagcgcaaccgcatgcacaacctaaacgccgcgctggacgcgctgcgcgaggtgctgcccaccttccccgaggatgccaagctcacgaagatcgagacgctgcgcttcgcccacaattacatctgggcgctcaccgagactctgcgcctggcggaccactgcgccggcgccggtggcctccagggggcgctcttcacggaggcggtgctcctgagcccgggagctgcgctcggcgccagcggggacagcccttctccaccttcctcctggagctgcaccaacagcccggcgtcatcctccaactccacgtccccatacagctgcactttatcgcccgctagccccgggtcagacgtggactactggcagcccccacctccggagaagcatcgttatgcgcctcacctgcccctcgccagggactgtatctag

SEQ ID NO: 3 - protein, 272 aa, Homo sapiens
MFVKSETLELKEEEDVLVLLGSASPALAALTPLSSSADEEEEEEPGASGGARRQRGAEAGQGARGGVAAGAEGCRPARLLGLVHDCKRRPSRARAVSRGAKTAETVQRIKKTRRLKANNRERNRMHNLNAALDALREVLPTFPEDAKLTKIETLRFAHNYIWALTETLRLADHCGGGGGGLPGALFSEAVLLSPGGASAALSSSGDSPSPASTWSCTNSPAPSSSVSSNSTSPYSCTLSPASPAGSDMDYWQPPPPDKHRYAPHLPIARDCI

SEQ ID NO: 4 - DNA, 819 bp, Homo sapiens
atgttcgtcaaatccgagaccttggagttgaaggaggaagaggacgtgttagtgctgctcggatcggcctcccccgccttggcggccctgaccccgctgtcatccagcgccgacgaagaagaggaggaggagccgggcgcgtcaggcggggcgcgtcggcagcgcggggctgaggccgggcagggggcgcggggcggcgtggctgcgggtgcggagggctgccggcccgcacggctgctgggtctggtacacgattgcaaacggcgcccttcccgggcgcgggccgtctcccgaggcgccaagacggccgagacggtgcagcgcatcaagaagacccgtagactgaaggccaacaaccgcgagcgaaaccgcatgcacaacctcaacgcggcactggacgcgctgcgcgaggtgctccccacgttccccgaggacgccaagctcaccaagatcgagaccctgcgcttcgcccacaactacatctgggcactcaccgagaccctgcgcctggcggatcactgcgggggcggcggcgggggcctgccgggggcgctcttctccgaggcagtgttgctgagcccgggaggagccagcgccgccctgagcagcagcggagacagcccctcgcccgcctccacgtggagttgcaccaacagccccgcgccgtcctcctccgtgtcctccaattccacctccccctacagctgcactttatcgcccgccagcccggccgggtcagacatggactattggcagcccccacctcccgacaagcaccgctatgcacctcacctccccatagccagggattgtatctag

SEQ ID NO: 5 - DNA, 1387 bp, Homo sapiens
ctctggtttcaagaccaatactcataacccccacatggaccaggcaccatcacacctgagcactgcacttagggtcaaagacctggccccacatctcagcagctatgtagactagctccagtcccttaatctctctcagcctcagtttcttcatctgcaaaacaggtctcagtttcgttgcaaagtatgaagtgctgggctgttactggtcaaagggaagagctgggaagagggtgcaaggtggggttgggctggagatgggctggagcagatagatggagggacctgaatggaggaagtaaaccaaggcccggtaacattgggactggacagagaacacgcagatcctctaggcaccggaagctaagtaacattgccctttctcctcctgtttgggactaggctgatgttgctgcctggaagggagccagcagaagggccccagcctgaagctgttaggtagaagccaaatccagggccagatttccaggaggcagcctcgggaagttgaaacacccggattcaggggtcaggaggcctgggcttctggcaccaaacggccagggacctactttccacctggagtcttgtaagagccactttcagcttgagctgcactttcgtcctccatgaaatgggggaggggatgctcctcacccaccttgcaaggttattttgaggcaaatgtcatggcgggactgagaattcttctgccctgcgaggaaatccagacatctctcccttacagacagggagactgaggtgaggcccttccaggcagagaaggtcactgttgcagccatgggcagtgccccacaggacctcgggtggtgcctctggagtctggagaagttcctaggggacctccgaggcaaagcagcccaaaagccgcctgtgagggtggctggtgtctgtccttcctcctaaggctggagtgtgcctgtggaggggtctcctgaactcccgcaaaggcagaaaggagggaagtaggggctgggacagttcatgcctcctccctgagggggtctcccgggctcggctcttggggccagagttcagggtgtctgggcctctctatgactttgttctaagtctttagggtggggctggggtctggcccagctgcaagggccccctcacccctgccccagagaggaacagccccgcacgggccctttaagaaggttgagggtgggggcaggtgggggagtccaagcctgaaacccgagcgggcgcgcgggtctgcgcctgccccgcccccggagttaagtgcgcggacacccggagccggcccgcgcccaggagcagagccgcgctcgctccactcagctcccagctcccaggactccgctggctcctcgcaagtcctgccgcccagcccgccggg

SEQ ID NO: 6 - DNA, 2209 bp, Homo sapiens
taatcccacctccctctctgtgctgggactcacagagggagacctcaggaggcagtctgtccatcacatgtccaaatgcagagcataccctgggctgggcgcagtggcgcacaactgtaattccagcactttgggaggctgatgtggaaggatcacttgagcccagaagttctagaccagcctgggcaacatggcaagaccctatctctacaaaaaaagttaaaaaatcagccacgtgtggtgacacacacctgtagtcccagctattcaggaggctgaggtgaggggatcacttaaggctgggaggttgaggctgcagtgagtcgtggttgcgccactgcactccagcctgggcaacagtgagaccctgtctcaaaagacaaaaaaaaaaaaaaaaaaaaaagaacatatcctggtgtggagtaggggacgctgctctgacagaggctcgggggcctgagctggctctgtgagctggggaggaggcagacagccaggccttgtctgcaagcagacctggcagcattgggctggccgccccccagggcctcctcttcatgcccagtgaatgactcaccttggcacagacacaatgttcggggtgggcacagtgcctgcttcccgccgcaccccagcccccctcaaatgccttccgagaagcccattgagcagggggcttgcattgcaccccagcctgacagcctggcatcttgggataaaagcagcacagccccctaggggctgcccttgctgtgtggcgccaccggcggtggagaacaaggctctattcagcctgtgcccaggaaaggggatcaggggatgcccaggcatggacagtgggtggcagggggggagaggagggctgtctgcttcccagaagtccaaggacacaaatgggtgaggggactgggcagggttctgaccctgtgggaccagagtggagggcgtagatggacctgaagtctccagggacaacagggcccaggtctcaggctcctagttgggcccagtggctccagcgtttccaaacccatccatccccagaggttcttcccatctctccaggctgatgtgtgggaactcgaggaaataaatctccagtgggagacggaggggtggccagggaaacggggcgctgcaggaataaagacgagccagcacagccagctcatgtgtaacggctttgtggagctgtcaaggcctggtctctgggagagaggcacagggaggccagacaaggaaggggtgacctggagggacagatccaggggctaaagtcctgataaggcaagagagtgccggccccctcttgccctatcaggacctccactgccacatagaggccatgattgacccttagacaaagggctggtgtccaatcccagcccccagccccagaactccagggaatgaatgggcagagagcaggaatgtgggacatctgtgttcaagggaaggactccaggagtctgctgggaatgaggcctagtaggaaatgaggtggcccttgagggtacagaacaggttcattcttcgccaaattcccagcaccttgcaggcacttacagctgagtgagataatgcctgggttatgaaatcaaaaagttggaaagcaggtcagaggtcatctggtacagcccttccttcccttttttttttttttttttgtgagacaaggtctctctctgttgcccaggctggagtggcgcaaacacagctcactgcagcctcaacctactgggctcaagcaatcctccagcctcagcctcccaaagtgctgggattacaagcatgagccaccccactcagccctttccttcctttttaattgatgcataataattgtaagtattcatcatggtccaaccaaccctttcttgacccaccttcctagagagagggtcctcttgcttcagcggtcagggccccagacccatggtctggctccaggtaccacctgcctcatgcaggagttggcgtgcccaggaagctctgcctctgggcacagtgacctcagtggggtgaggggagctctccccatagctgggctgcggcccaaccccaccccctcaggctatgccagggggtgttgccaggggcacccgggcatcgccagtctagcccactccttcataaagccctcgcatcccaggagcgagcagagccagagcaggttggagaggagacgcatcacctccgctgctcgcgg